European Patent Specification EP 4 056 698 B1, published January 3, 2024. Title: Novel urease accessory protein variant and a method for producing L-valine using the same. Applicant: CJ CheilJedang Corporation. The sequence listing filed with the application follows.

SEQUENCE LISTING (11 sequences)

SEQ ID NO: 1 - protein, 157 aa, Artificial Sequence
  Urease accessory protein variant
MIITAIDTNIYDQPEFVEGRDVIGVRFEDLVLDKRIQRVALSGGEELGLRLNHGHLILREGDVLKADDKTVFVVEIIPTDVLVITPSDIHQMGFVAHSLGNRHLPAQFSKPGEVTEKAAMIVQYDHTVVSFLDEHSIEYQRTELVPPIPFRHSGHTH

SEQ ID NO: 2 - DNA, 474 bp, Artificial Sequence
  Urease accessory protein variant coding gene
atgattatcactgcgatcgacaccaacatctacgatcaaccggagtttgttgaaggacgcgatgtcatcggtgtgcgttttgaagatttagtgctggataagcgcattcaacgtgttgcgctctccggaggagaagaactggggttgcggctcaatcacgggcacctcatcctgcgggaaggcgatgtgctgaaagccgatgataagacagtatttgtggtggagattattcccacggatgttttagtcatcacaccaagcgatattcaccagatgggatttgtggcgcactctctgggaaataggcatctgccagcacagttttccaagccaggtgaagtgacagagaaggcagccatgatcgtgcaatacgatcacacggtggtcagcttcttagatgagcacagcattgagtatcagcgcaccgaacttgttccgccaattcctttcaggcatagcgggcacacacattga

SEQ ID NO: 3 - protein, 157 aa, Artificial Sequence
  Wild-type urease accessory protein
MIITAIDTNIYDQPEFVEGRDVIGVRFEDLVLDKRIQRVALSGGEELGLRLNHGHPILREGDVLKADDKTVFVVEIIPTDVLVITPSDIHQMGFVAHSLGNRHLPAQFSKPGEVTEKAAMIVQYDHTVVSFLDEHSIEYQRTELVPPIPFRHSGHTH

SEQ ID NO: 4 - DNA, 474 bp, Artificial Sequence
  Wild-type urease accessory protein coding gene
atgattatcactgcgatcgacaccaacatctacgatcaaccggagtttgttgaaggacgcgatgtcatcggtgtgcgttttgaagatttagtgctggataagcgcattcaacgtgttgcgctctccggaggagaagaactggggttgcggctcaatcacgggcaccccatcctgcgggaaggcgatgtgctgaaagccgatgataagacagtatttgtggtggagattattcccacggatgttttagtcatcacaccaagcgatattcaccagatgggatttgtggcgcactctctgggaaataggcatctgccagcacagttttccaagccaggtgaagtgacagagaaggcagccatgatcgtgcaatacgatcacacggtggtcagcttcttagatgagcacagcattgagtatcagcgcaccgaacttgttccgccaattcctttcaggcatagcgggcacacacattga

SEQ ID NO: 5 - DNA, 36 bp, Artificial Sequence
  ureE_1F
tcgagctcggtaccctgggttgatggtcaattccct

SEQ ID NO: 6 - DNA, 44 bp, Artificial Sequence
  ureE_2R
cacatcgccttcccgcaggatgaggtgcccgtgattgagccgca

SEQ ID NO: 7 - DNA, 44 bp, Artificial Sequence
  ureE_3F
tgcggctcaatcacgggcacctcatcctgcgggaaggcgatgtg

SEQ ID NO: 8 - DNA, 36 bp, Artificial Sequence
  ureE_4R
ctctagaggatccccaaacatcctcattgccaaagc

SEQ ID NO: 9 - DNA, 21 bp, Artificial Sequence
  ureE_5F
tgggttgatggtcaattccct

SEQ ID NO: 10 - DNA, 21 bp, Artificial Sequence
  ureE_6R
aaacatcctcattgccaaagc

SEQ ID NO: 11 - DNA, 5803 bp, Artificial Sequence
  pDCM2
gttcgcttgctgtccataaaaccgcccagtctagctatcgccatgtaagcccactgcaagctacctgctttctctttgcgcttgcgttttcccttgtccagatagcccagtagctgacattcatccggggtcagcaccgtttctgcggactggctttctacgtgttccgcttcctttagcagcccttgcgccctgagtgcttgcggcagcgtgaagctagcttttatcgccattcgccattcaggctgcgcaactgttgggaagggcgatcggtgcgggcctcttcgctattacgccagctggcgaaagggggatgtgctgcaaggcgattaagttgggtaacgccagggttttcccagtcacgacgttgtaaaacgacggccagtgaattcgagctcggtacccggggatcctctagagtcgacctgcaggcatgcaagcttggcgtaatcatggtcatagctgtttcctgtgtgaaattgttatccgctcacaattccacacaacatacgagccggaagcataaagtgtaaagcctggggtgcctaatgagtgagctaactcacattaattgcgttgcgctcactgcccgctttccagtcgggaaacctgtcgtgccagctgcattaatgaatcggccaacgcgcggggagaggcggtttgcgtattgggcgctcttccgcttcctcgctcactgactcgctgcgctcggtcgttcggctgcggcgagcggtatcagctcactcaaaggcggtaatacggttatccacagaatcaggggataacgcaggaaagaacatgtgagcaaaaggccagcaaaaggccaggaaccgtaaaaaggccgcgttgctggcgtttttccataggctccgcccccctgacgagcatcacaaaaatcgacgctcaagtcagaggtggcgaaacccgacaggactataaagataccaggcgtttccccctggaagctccctcgtgcgctctcctgttccgaccctgccgcttaccggatacctgtccgcctttctcccttcgggaagcgtggcgctttctcaatgctcacgctgtaggtatctcagttcggtgtaggtcgttcgctccaagctgggctgtgtgcacgaaccccccgttcagcccgaccgctgcgccttatccggtaactatcgtcttgagtccaacccggtaagacacgacttatcgccactggcagcagccactggtaacaggattagcagagcgaggtatgtaggcggtgctacagagttcttgaagtggtggcctaactacggctacactagaaggacagtatttggtatctgcgctctgctgaagccagttaccttcggaaaaagagttggtagctcttgatccggcaaacaaaccaccgctggtagcggtggtttttttgtttgcaagcagcagattacgcgcagaaaaaaaggatctcaagaagatcctttgatcttttctacggggtctgacgctcagtggaacgaaaactcacgttaagggattttggtcatgagattatcaaaaaggatcttcacctagatccttttggggtgggcgaagaactccagcatgagatccccgcgctggaggatcatccagccctgatagaaacagaagccactggagcacctcaaaaacaccatcatacactaaatcagtaagttggcagcatcacccgacgcactttgcgccgaataaatacctgtgacggaagatcacttcgcagaataaataaatcctggtgtccctgttgataccgggaagccctgggccaacttttggcgaaaatgagacgttgatcggcacgtaagaggttccaactttcaccataatgaaataagatcactaccgggcgtattttttgagttatcgagattttcaggagctgatagaaacagaagccactggagcacctcaaaaacaccatcatacactaaatcagtaagttggcagcatcacccgacgcactttgcgccgaataaatacctgtgacggaagatcacttcgcagaataaataaatcctggtgtccctgttgataccgggaagccctgggccaacttttggcgaaaatgagacgttgatcggcacgtaagaggttccaactttcaccataatgaaataagatcactaccgggcgtattttttgagttatcgagattttcaggagctctttggcatcgtctctcgcctgtcccctcagttcagtaatttcctgcatttgcctgtttccagtcggtagatattccacaaaacagcagggaagcagcgcttttccgctgcataaccctgcttcggggtcattatagcgattttttcggtatatccatcctttttcgcacgatatacaggattttgccaaagggttcgtgtagactttccttggtgtatccaacggcgtcagccgggcaggataggtgaagtaggcccacccgcgagcgggtgttccttcttcactgtcccttattcgcacctggcggtgctcaacgggaatcctgctctgcgaggctggccggctaccgccggcgtaacagatgagggcaagcggatggctgatgaaaccaagccaaccaggaagggcagcccacctatcaaggtgtactgccttccagacgaacgaagagcgattgaggaaaaggcggcggcggccggcatgagcctgtcggcctacctgctggccgtcggccagggctacaaaatcacgggcgtcgtggactatgagcacgtccgcgagggcgtcccggaaaacgattccgaagcccaacctttcatagaaggcggcggtggaatcgaaatctcgtgatggcaggttgggcgtcgcttggtcggtcatttcgaaaaaggttaggaatacggttagccatttgcctgcttttatatagttcantatgggattcacctttatgttgataagaaataaaagaaaatgccaataggatatcggcattttcttttgcgtttttatttgttaactgttaattgtccttgttcaaggatgctgtctttgacaacagatgttttcttgcctttgatgttcagcaggaagctcggcgcaaacgttgattgtttgtctgcgtagaatcctctgtttgtcatatagcttgtaatcacgacattgtttcctttcgcttgaggtacagcgaagtgtgagtaagtaaaggttacatcgttaggcggatcaagatccatttttaacacaaggccagttttgttcagcggcttgtatgggccagttaaagaattagaaacataaccaagcatgtaaatatcgttagacgtaatgccgtcaatcgtcatttttgatccgcgggagtcagtgaacaggtaccatttgccgttcattttaaagacgttcgcgcgttcaatttcatctgttactgtgttagatgcaatcagcggtttcatcacttttttcagtgtgtaatcatcgtttagctcaatcataccgagagcgccgtttgctaactcagccgtgcgttttttatcgctttgcagaagtttttgactttcttgacggaagaatgatgtgcttttgccatagtatgctttgttaaataaagattcttcgccttggtagccatcttcagttccagtgtttgcttcaaatactaagtatttgtggcctttatcttctacgtagtgaggatctctcagcgtatggttgtcgcctgagctgtagttgccttcatcgatgaactgctgtacattttgatacgtttttccgtcaccgtcaaagattgatttataatcctctacaccgttgatgttcaaagagctgtctgatgctgatacgttaacttgtgcagttgtcagtgtttgtttgccgtaatgtttaccggagaaatcagtgtagaataaacggatttttccgtcagatgtaaatgtggctgaacctgaccattcttgtgtttggtcttttaggatagaatcatttgcatcgaatttgtcgctgtctttaaagacgcggccagcgtttttccagctgtcaatagaagtttcgccgactttttgatagaacatgtaaatcgatgtgtcatccgcatttttaggatctccggctaatgcaaagacgatgtggtagccgtgatagtttgcgacagtgccgtcagcgttttgtaatggccagctgtcccaaacgtccaggccttttgcagaagagatatttttaattgtggacgaatcaaattcagaaacttgatatttttcatttttttgctgttcagggatttgcagcatatcatggcgtgtaatatgggaaatgccgtatgtttccttatatggcttttggttcgtttctttcgcaaacgcttgagttgcgcctcctgccagcagtgcggtagtaaaggttaatactgttgcttgttttgcaaactttttgatgttcatcgttcatgtctccttttttatgtactgtgttagcggtctgcttcttccagccctcctgtttgaagatggcaagttagttacgcacaataaaaaaagacctaaaatatgtaaggggtgacgccaaagtatacactttgccctttacacattttaggtcttgcctgctttatcagtaacaaacccgcgcgatttacttttcgacctcattctattagactctcgtttggattgcaactggtctattttcctcttttgtttgatagaaaatcataaaaggatttgcagactacgggcctaaagaactaaaaaatctatctgtttcttttcattctctgtattttttatagtttctgttgcatgggcataaagttgcctttttaatcacaattcagaaaatatcataatatctcatttcactaaataatagtgaacggcaggtatatgtgatgggttaaaaaggatcaccccagagtcccgctcagaagaactcgtcaagaaggcgatagaaggcgatgcgctgcgaatcgggagcggcgataccgtaaagcacgaggaagcggtcagcccattcgccgccaagctcttcagcaatatcacgggtagccaacgctatgtcctgatagcggtccgccacacccagccggccacagtcgatgaatccagaaaagcggccattttccaccatgatattcggcaagcaggcatcgccatgggtcacgacgagatcctcgccgtcgggcatccgcgccttgagcctggcgaacagttcggctggcgcgagcccctgatgctcttcgtccagatcatcctgatcgacaagaccggcttccatccgagtacgtgctcgctcgatgcgatgtttcgcttggtggtcgaatgggcaggtagccggatcaagcgtatgcagccgccgcattgcatcagccatgatggatactttctcggcaggagcaaggtgagatgacaggagatcctgccccggcacttcgcccaatagcagccagtcccttcccgcttcagtgacaacgtcgagacagctgcgcaaggaacgcccgtcgtggccagccacgatagccgcgctgcctcgtcttggagttcattcagggcaccggacaggtcggtcttgacaaaaagaaccgggcgcccctgcgctgacagccggaacacggcggcatcagagcagccgattgtctgttgtgcccagtcatagccgaatagcctctccacccaagcggccggagaacctgcgtgcaatccatcttgttcaatcatgcgaaacgatcctcatcctgtctcttgatcagatcttgatcccctgcgccatcagatccttggcggcaagaaagccatccagtttactttgcagggcttcccaaccttaccagagggcgccccagctggcaattccg